European Patent Application EP 4 176 889 A1, published May 10, 2023. Title: Composition for promoting intestinal development, improving lung function, and  improving  immunity. Applicant: Morinaga Milk Industry Co., Ltd. The sequence listing filed with the application follows.

SEQUENCE LISTING (12 sequences)

SEQ ID NO: 1 - DNA, 18 bp, Artificial Sequence
  G3PDH Fwd
cctcccgcttcgctctct

SEQ ID NO: 2 - DNA, 17 bp, Artificial Sequence
  G3PDH Rev
gctggcgacgcaaaaga

SEQ ID NO: 3 - DNA, 20 bp, Artificial Sequence
  IL-6 Fwd
tggataagctgcagtcacag

SEQ ID NO: 4 - DNA, 20 bp, Artificial Sequence
  IL-6 Rev
attatccgaatggccctcag

SEQ ID NO: 5 - DNA, 21 bp, Artificial Sequence
  IL-8 Fwd
gctctctgtgaggctgcagtt

SEQ ID NO: 6 - DNA, 22 bp, Artificial Sequence
  IL-8  Rev
tttatgcactggcatcgaagtt

SEQ ID NO: 7 - DNA, 23 bp, Artificial Sequence
  MCP-1 Fwd
acagaaagagtcaccagcagcaa

SEQ ID NO: 8 - DNA, 16 bp, Artificial Sequence
  MCP-1 Rev
gcccgcgatggtcttg

SEQ ID NO: 9 - DNA, 20 bp, Artificial Sequence
  IFN- À Fwd
agttgcctgggactcctcaa

SEQ ID NO: 10 - DNA, 22 bp, Artificial Sequence
  IFN- À Rev
cctcagggacctcaaagttcat

SEQ ID NO: 11 - DNA, 23 bp, Artificial Sequence
  IFN- Á Fwd
tggtagctctgggaaactgaatg

SEQ ID NO: 12 - DNA, 18 bp, Artificial Sequence
  IFN- Á Rev
ggctttgcgctggatctg